European Patent Application EP 4 527 927 A1, published March 26, 2025. Title: Oligonucleotide-based strategies to combat respiratory viruses. Applicant: Medizinische Hochschule Hannover. The sequence listing filed with the application follows.

SEQUENCE LISTING (206 sequences)

SEQ ID NO: 1 - RNA, 22 nt, synthetic construct
  source 1..22: mol_type = other RNA
ttaattttctaatagatcgttg

SEQ ID NO: 2 - RNA, 22 nt, synthetic construct
  source 1..22: mol_type = other RNA
ttacaaaacatcttgacatggc

SEQ ID NO: 3 - RNA, 22 nt, synthetic construct
  source 1..22: mol_type = other RNA
tatatgaacatcttgctactta

SEQ ID NO: 4 - RNA, 22 nt, synthetic construct
  source 1..22: mol_type = other RNA
taaaacaacatcatcatcccca

SEQ ID NO: 5 - RNA, 22 nt, synthetic construct
  source 1..22: mol_type = other RNA
tttgataaaacaacttcactgg

SEQ ID NO: 6 - RNA, 22 nt, synthetic construct
  source 1..22: mol_type = other RNA
tatcaataagaaatccttctgg

SEQ ID NO: 7 - RNA, 22 nt, synthetic construct
  source 1..22: mol_type = other RNA
ttaataaatcttttaatatcag

SEQ ID NO: 8 - RNA, 22 nt, synthetic construct
  source 1..22: mol_type = other RNA
ttaagtaataattcagtcactt

SEQ ID NO: 9 - RNA, 22 nt, synthetic construct
  source 1..22: mol_type = other RNA
tcaaatatcaattccatctcgg

SEQ ID NO: 10 - RNA, 22 nt, synthetic construct
  source 1..22: mol_type = other RNA
tttataaactatctccttctta

SEQ ID NO: 11 - RNA, 22 nt, synthetic construct
  source 1..22: mol_type = other RNA
taatattaaaaccaattctgga

SEQ ID NO: 12 - RNA, 22 nt, synthetic construct
  source 1..22: mol_type = other RNA
tatatatagatcttgttaccta

SEQ ID NO: 13 - RNA, 22 nt, synthetic construct
  source 1..22: mol_type = other RNA
tattattgttcttaaatcttgt

SEQ ID NO: 14 - RNA, 22 nt, synthetic construct
  source 1..22: mol_type = other RNA
tcttatatcactgtaatcagta

SEQ ID NO: 15 - RNA, 22 nt, synthetic construct
  source 1..22: mol_type = other RNA
tagatcattaatattatccgat

SEQ ID NO: 16 - RNA, 22 nt, synthetic construct
  source 1..22: mol_type = other RNA
ttttattcttatatcactgtaa

SEQ ID NO: 17 - RNA, 22 nt, synthetic construct
  source 1..22: mol_type = other RNA
ttttaatatctaatgatctata

SEQ ID NO: 18 - RNA, 22 nt, synthetic construct
  source 1..22: mol_type = other RNA
tctaatgatctatagatctgtc

SEQ ID NO: 19 - RNA, 22 nt, synthetic construct
  source 1..22: mol_type = other RNA
tttgtttgttaatacatatggt

SEQ ID NO: 20 - RNA, 22 nt, synthetic construct
  source 1..22: mol_type = other RNA
tttaatatctaatgatctatag

SEQ ID NO: 21 - RNA, 22 nt, synthetic construct
  source 1..22: mol_type = other RNA
tagatcataaatatcatattta

SEQ ID NO: 22 - RNA, 22 nt, synthetic construct
  source 1..22: mol_type = other RNA
ttagtaattgttaacatcttca

SEQ ID NO: 23 - RNA, 22 nt, synthetic construct
  source 1..22: mol_type = other RNA
taacatttcattttgtatctgt

SEQ ID NO: 24 - RNA, 22 nt, synthetic construct
  source 1..22: mol_type = other RNA
ttaacatttcattttgtatctg

SEQ ID NO: 25 - RNA, 22 nt, synthetic construct
  source 1..22: mol_type = other RNA
ttgtatgaacttaatatctctg

SEQ ID NO: 26 - RNA, 22 nt, synthetic construct
  source 1..22: mol_type = other RNA
tttgattttctatcaatcttct

SEQ ID NO: 27 - RNA, 22 nt, synthetic construct
  source 1..22: mol_type = other RNA
taaacaatcatttctttcgctt

SEQ ID NO: 28 - RNA, 22 nt, synthetic construct
  source 1..22: mol_type = other RNA
ttgattgatattgtgctgggta

SEQ ID NO: 29 - RNA, 22 nt, synthetic construct
  source 1..22: mol_type = other RNA
ttaggaattttgaacaaggtta

SEQ ID NO: 30 - RNA, 22 nt, synthetic construct
  source 1..22: mol_type = other RNA
taagaagacatccaaataccgg

SEQ ID NO: 31 - RNA, 22 nt, synthetic construct
  source 1..22: mol_type = other RNA
taaatatgtacaaatatctgga

SEQ ID NO: 32 - RNA, 22 nt, synthetic construct
  source 1..22: mol_type = other RNA
ttaatttccaaaattataccta

SEQ ID NO: 33 - RNA, 22 nt, synthetic construct
  source 1..22: mol_type = other RNA
ttatgaatcaagaaccaggtga

SEQ ID NO: 34 - RNA, 22 nt, synthetic construct
  source 1..22: mol_type = other RNA
tatagtttaaaaatagaaggta

SEQ ID NO: 35 - RNA, 22 nt, synthetic construct
  source 1..22: mol_type = other RNA
tagattagaagaaaccacagga

SEQ ID NO: 36 - RNA, 22 nt, synthetic construct
  source 1..22: mol_type = other RNA
taattcaaactcatgatcctgt

SEQ ID NO: 37 - RNA, 22 nt, synthetic construct
  source 1..22: mol_type = other RNA
taaaattaacaatttctgggga

SEQ ID NO: 38 - RNA, 22 nt, synthetic construct
  source 1..22: mol_type = other RNA
ttagattagaagaaaccacagg

SEQ ID NO: 39 - RNA, 22 nt, synthetic construct
  source 1..22: mol_type = other RNA
tagtaaatcaatttgcatacac

SEQ ID NO: 40 - RNA, 22 nt, synthetic construct
  source 1..22: mol_type = other RNA
ttcaaattacatatacctggta

SEQ ID NO: 41 - RNA, 22 nt, synthetic construct
  source 1..22: mol_type = other RNA
atctattgaaacaatatcttga

SEQ ID NO: 42 - RNA, 22 nt, synthetic construct
  source 1..22: mol_type = other RNA
ttcattgtcattatcgactcga

SEQ ID NO: 43 - RNA, 22 nt, synthetic construct
  source 1..22: mol_type = other RNA
tacatcaacaaatttatcacac

SEQ ID NO: 44 - RNA, 22 nt, synthetic construct
  source 1..22: mol_type = other RNA
tattaatgatctaatacagtca

SEQ ID NO: 45 - RNA, 22 nt, synthetic construct
  source 1..22: mol_type = other RNA
taatgatctaatacagtcagga

SEQ ID NO: 46 - RNA, 22 nt, synthetic construct
  source 1..22: mol_type = other RNA
ttatcaatagtcttcatcatag

SEQ ID NO: 47 - RNA, 22 nt, synthetic construct
  source 1..22: mol_type = other RNA
ttcaaaagagaaatcgagtgga

SEQ ID NO: 48 - RNA, 22 nt, synthetic construct
  source 1..22: mol_type = other RNA
taaacaattctgttgcacttga

SEQ ID NO: 49 - RNA, 22 nt, synthetic construct
  source 1..22: mol_type = other RNA
ttaagattacagaaggatgtga

SEQ ID NO: 50 - RNA, 22 nt, synthetic construct
  source 1..22: mol_type = other RNA
tatgtcaacaaagaaatcgtgc

SEQ ID NO: 51 - RNA, 22 nt, synthetic construct
  source 1..22: mol_type = other RNA
tataaaaccagaactgtaccca

SEQ ID NO: 52 - RNA, 22 nt, synthetic construct
  source 1..22: mol_type = other RNA
taaatcaactaatatctcctcg

SEQ ID NO: 53 - RNA, 22 nt, synthetic construct
  source 1..22: mol_type = other RNA
tactaatgaaaaatagtaggat

SEQ ID NO: 54 - RNA, 22 nt, synthetic construct
  source 1..22: mol_type = other RNA
ttaagaaatcaagagatactga

SEQ ID NO: 55 - RNA, 22 nt, synthetic construct
  source 1..22: mol_type = other RNA
tcatacaaaagaatcaatccga

SEQ ID NO: 56 - RNA, 22 nt, synthetic construct
  source 1..22: mol_type = other RNA
tactaaacaatgtagatactgc

SEQ ID NO: 57 - DNA, 67 bp, synthetic construct
  source 1..67: mol_type = other DNA
agcgaaacgatctattagaaaattaatagtgaagccacagatgtattaattttctaatagatcgttg

SEQ ID NO: 58 - DNA, 67 bp, synthetic construct
  source 1..67: mol_type = other DNA
ggcacaacgatctattagaaaattaatacatctgtggcttcactattaattttctaatagatcgttt

SEQ ID NO: 59 - DNA, 67 bp, synthetic construct
  source 1..67: mol_type = other DNA
agcgaccatgtcaagatgttttgtaatagtgaagccacagatgtattacaaaacatcttgacatggc

SEQ ID NO: 60 - DNA, 67 bp, synthetic construct
  source 1..67: mol_type = other DNA
ggcagccatgtcaagatgttttgtaatacatctgtggcttcactattacaaaacatcttgacatggt

SEQ ID NO: 61 - DNA, 67 bp, synthetic construct
  source 1..67: mol_type = other DNA
agcgcaagtagcaagatgttcatatatagtgaagccacagatgtatatatgaacatcttgctactta

SEQ ID NO: 62 - DNA, 67 bp, synthetic construct
  source 1..67: mol_type = other DNA
ggcataagtagcaagatgttcatatatacatctgtggcttcactatatatgaacatcttgctacttg

SEQ ID NO: 63 - DNA, 67 bp, synthetic construct
  source 1..67: mol_type = other DNA
agcgcggggatgatgatgttgttttatagtgaagccacagatgtataaaacaacatcatcatcccca

SEQ ID NO: 64 - DNA, 67 bp, synthetic construct
  source 1..67: mol_type = other DNA
ggcatggggatgatgatgttgttttatacatctgtggcttcactataaaacaacatcatcatccccg

SEQ ID NO: 65 - DNA, 67 bp, synthetic construct
  source 1..67: mol_type = other DNA
agcgacagtgaagttgttttatcaaatagtgaagccacagatgtatttgataaaacaacttcactgg

SEQ ID NO: 66 - DNA, 67 bp, synthetic construct
  source 1..67: mol_type = other DNA
ggcaccagtgaagttgttttatcaaatacatctgtggcttcactatttgataaaacaacttcactgt

SEQ ID NO: 67 - DNA, 67 bp, synthetic construct
  source 1..67: mol_type = other DNA
agcgacagaaggatttcttattgatatagtgaagccacagatgtatatcaataagaaatccttctgg

SEQ ID NO: 68 - DNA, 67 bp, synthetic construct
  source 1..67: mol_type = other DNA
ggcaccagaaggatttcttattgatatacatctgtggcttcactatatcaataagaaatccttctgt

SEQ ID NO: 69 - DNA, 67 bp, synthetic construct
  source 1..67: mol_type = other DNA
agcgatgatattaaaagatttattaatagtgaagccacagatgtattaataaatcttttaatatcag

SEQ ID NO: 70 - DNA, 67 bp, synthetic construct
  source 1..67: mol_type = other DNA
ggcactgatattaaaagatttattaatacatctgtggcttcactattaataaatcttttaatatcat

SEQ ID NO: 71 - DNA, 67 bp, synthetic construct
  source 1..67: mol_type = other DNA
agcgcagtgactgaattattacttaatagtgaagccacagatgtattaagtaataattcagtcactt

SEQ ID NO: 72 - DNA, 67 bp, synthetic construct
  source 1..67: mol_type = other DNA
ggcaaagtgactgaattattacttaatacatctgtggcttcactattaagtaataattcagtcactg

SEQ ID NO: 73 - DNA, 67 bp, synthetic construct
  source 1..67: mol_type = other DNA
agcgacgagatggaattgatatttgatagtgaagccacagatgtatcaaatatcaattccatctcgg

SEQ ID NO: 74 - DNA, 67 bp, synthetic construct
  source 1..67: mol_type = other DNA
ggcaccgagatggaattgatatttgatacatctgtggcttcactatcaaatatcaattccatctcgt

SEQ ID NO: 75 - DNA, 67 bp, synthetic construct
  source 1..67: mol_type = other DNA
agcgcaagaaggagatagtttataaatagtgaagccacagatgtatttataaactatctccttctta

SEQ ID NO: 76 - DNA, 67 bp, synthetic construct
  source 1..67: mol_type = other DNA
ggcataagaaggagatagtttataaatacatctgtggcttcactatttataaactatctccttcttg

SEQ ID NO: 77 - DNA, 67 bp, synthetic construct
  source 1..67: mol_type = other DNA
agcgcccagaattggttttaatattatagtgaagccacagatgtataatattaaaaccaattctgga

SEQ ID NO: 78 - DNA, 67 bp, synthetic construct
  source 1..67: mol_type = other DNA
ggcatccagaattggttttaatattatacatctgtggcttcactataatattaaaaccaattctggg

SEQ ID NO: 79 - DNA, 67 bp, synthetic construct
  source 1..67: mol_type = other DNA
agcgcaggtaacaagatctatatatatagtgaagccacagatgtatatatatagatcttgttaccta

SEQ ID NO: 80 - DNA, 67 bp, synthetic construct
  source 1..67: mol_type = other DNA
ggcataggtaacaagatctatatatatacatctgtggcttcactatatatatagatcttgttacctg

SEQ ID NO: 81 - DNA, 67 bp, synthetic construct
  source 1..67: mol_type = other DNA
agcgccaagatttaagaacaataatatagtgaagccacagatgtatattattgttcttaaatcttgt

SEQ ID NO: 82 - DNA, 67 bp, synthetic construct
  source 1..67: mol_type = other DNA
ggcaacaagatttaagaacaataatatacatctgtggcttcactatattattgttcttaaatcttgg

SEQ ID NO: 83 - DNA, 67 bp, synthetic construct
  source 1..67: mol_type = other DNA
agcgcactgattacagtgatataagatagtgaagccacagatgtatcttatatcactgtaatcagta

SEQ ID NO: 84 - DNA, 67 bp, synthetic construct
  source 1..67: mol_type = other DNA
ggcatactgattacagtgatataagatacatctgtggcttcactatcttatatcactgtaatcagtg

SEQ ID NO: 85 - DNA, 67 bp, synthetic construct
  source 1..67: mol_type = other DNA
agcgctcggataatattaatgatctatagtgaagccacagatgtatagatcattaatattatccgat

SEQ ID NO: 86 - DNA, 67 bp, synthetic construct
  source 1..67: mol_type = other DNA
ggcaatcggataatattaatgatctatacatctgtggcttcactatagatcattaatattatccgag

SEQ ID NO: 87 - DNA, 67 bp, synthetic construct
  source 1..67: mol_type = other DNA
agcgctacagtgatataagaataaaatagtgaagccacagatgtattttattcttatatcactgtaa

SEQ ID NO: 88 - DNA, 67 bp, synthetic construct
  source 1..67: mol_type = other DNA
ggcattacagtgatataagaataaaatacatctgtggcttcactattttattcttatatcactgtag

SEQ ID NO: 89 - DNA, 67 bp, synthetic construct
  source 1..67: mol_type = other DNA
agcgcatagatcattagatattaaaatagtgaagccacagatgtattttaatatctaatgatctata

SEQ ID NO: 90 - DNA, 67 bp, synthetic construct
  source 1..67: mol_type = other DNA
ggcatatagatcattagatattaaaatacatctgtggcttcactattttaatatctaatgatctatg

SEQ ID NO: 91 - DNA, 67 bp, synthetic construct
  source 1..67: mol_type = other DNA
agcgaacagatctatagatcattagatagtgaagccacagatgtatctaatgatctatagatctgtc

SEQ ID NO: 92 - DNA, 67 bp, synthetic construct
  source 1..67: mol_type = other DNA
ggcagacagatctatagatcattagatacatctgtggcttcactatctaatgatctatagatctgtt

SEQ ID NO: 93 - DNA, 67 bp, synthetic construct
  source 1..67: mol_type = other DNA
agcgcccatatgtattaacaaacaaatagtgaagccacagatgtatttgtttgttaatacatatggt

SEQ ID NO: 94 - DNA, 67 bp, synthetic construct
  source 1..67: mol_type = other DNA
ggcaaccatatgtattaacaaacaaatacatctgtggcttcactatttgtttgttaatacatatggg

SEQ ID NO: 95 - DNA, 67 bp, synthetic construct
  source 1..67: mol_type = other DNA
agcgatatagatcattagatattaaatagtgaagccacagatgtatttaatatctaatgatctatag

SEQ ID NO: 96 - DNA, 67 bp, synthetic construct
  source 1..67: mol_type = other DNA
ggcactatagatcattagatattaaatacatctgtggcttcactatttaatatctaatgatctatat

SEQ ID NO: 97 - DNA, 67 bp, synthetic construct
  source 1..67: mol_type = other DNA
agcgcaaatatgatatttatgatctatagtgaagccacagatgtatagatcataaatatcatattta

SEQ ID NO: 98 - DNA, 67 bp, synthetic construct
  source 1..67: mol_type = other DNA
ggcataaatatgatatttatgatctatacatctgtggcttcactatagatcataaatatcatatttg

SEQ ID NO: 99 - DNA, 67 bp, synthetic construct
  source 1..67: mol_type = other DNA
agcgcgaagatgttaacaattactaatagtgaagccacagatgtattagtaattgttaacatcttca

SEQ ID NO: 100 - DNA, 67 bp, synthetic construct
  source 1..67: mol_type = other DNA
ggcatgaagatgttaacaattactaatacatctgtggcttcactattagtaattgttaacatcttcg

SEQ ID NO: 101 - DNA, 67 bp, synthetic construct
  source 1..67: mol_type = other DNA
agcgccagatacaaaatgaaatgttatagtgaagccacagatgtataacatttcattttgtatctgt

SEQ ID NO: 102 - DNA, 67 bp, synthetic construct
  source 1..67: mol_type = other DNA
ggcaacagatacaaaatgaaatgttatacatctgtggcttcactataacatttcattttgtatctgg

SEQ ID NO: 103 - DNA, 67 bp, synthetic construct
  source 1..67: mol_type = other DNA
agcgaagatacaaaatgaaatgttaatagtgaagccacagatgtattaacatttcattttgtatctg

SEQ ID NO: 104 - DNA, 67 bp, synthetic construct
  source 1..67: mol_type = other DNA
ggcacagatacaaaatgaaatgttaatacatctgtggcttcactattaacatttcattttgtatctt

SEQ ID NO: 105 - DNA, 67 bp, synthetic construct
  source 1..67: mol_type = other DNA
agcgaagagatattaagttcatacaatagtgaagccacagatgtattgtatgaacttaatatctctg

SEQ ID NO: 106 - DNA, 67 bp, synthetic construct
  source 1..67: mol_type = other DNA
ggcacagagatattaagttcatacaatacatctgtggcttcactattgtatgaacttaatatctctt

SEQ ID NO: 107 - DNA, 67 bp, synthetic construct
  source 1..67: mol_type = other DNA
agcgcgaagattgatagaaaatcaaatagtgaagccacagatgtatttgattttctatcaatcttct

SEQ ID NO: 108 - DNA, 67 bp, synthetic construct
  source 1..67: mol_type = other DNA
ggcaagaagattgatagaaaatcaaatacatctgtggcttcactatttgattttctatcaatcttcg

SEQ ID NO: 109 - DNA, 67 bp, synthetic construct
  source 1..67: mol_type = other DNA
agcgcagcgaaagaaatgattgtttatagtgaagccacagatgtataaacaatcatttctttcgctt

SEQ ID NO: 110 - DNA, 67 bp, synthetic construct
  source 1..67: mol_type = other DNA
ggcaaagcgaaagaaatgattgtttatacatctgtggcttcactataaacaatcatttctttcgctg

SEQ ID NO: 111 - DNA, 67 bp, synthetic construct
  source 1..67: mol_type = other DNA
agcgcacccagcacaatatcaatcaatagtgaagccacagatgtattgattgatattgtgctgggta

SEQ ID NO: 112 - DNA, 67 bp, synthetic construct
  source 1..67: mol_type = other DNA
ggcatacccagcacaatatcaatcaatacatctgtggcttcactattgattgatattgtgctgggtg

SEQ ID NO: 113 - DNA, 67 bp, synthetic construct
  source 1..67: mol_type = other DNA
agcgcaaccttgttcaaaattcctaatagtgaagccacagatgtattaggaattttgaacaaggtta

SEQ ID NO: 114 - DNA, 67 bp, synthetic construct
  source 1..67: mol_type = other DNA
ggcataaccttgttcaaaattcctaatacatctgtggcttcactattaggaattttgaacaaggttg

SEQ ID NO: 115 - DNA, 67 bp, synthetic construct
  source 1..67: mol_type = other DNA
agcgacggtatttggatgtcttcttatagtgaagccacagatgtataagaagacatccaaataccgg

SEQ ID NO: 116 - DNA, 67 bp, synthetic construct
  source 1..67: mol_type = other DNA
ggcaccggtatttggatgtcttcttatacatctgtggcttcactataagaagacatccaaataccgt

SEQ ID NO: 117 - DNA, 67 bp, synthetic construct
  source 1..67: mol_type = other DNA
agcgcccagatatttgtacatatttatagtgaagccacagatgtataaatatgtacaaatatctgga

SEQ ID NO: 118 - DNA, 67 bp, synthetic construct
  source 1..67: mol_type = other DNA
ggcatccagatatttgtacatatttatacatctgtggcttcactataaatatgtacaaatatctggg

SEQ ID NO: 119 - DNA, 67 bp, synthetic construct
  source 1..67: mol_type = other DNA
agcgcaggtataattttggaaattaatagtgaagccacagatgtattaatttccaaaattataccta

SEQ ID NO: 120 - DNA, 67 bp, synthetic construct
  source 1..67: mol_type = other DNA
ggcataggtataattttggaaattaatacatctgtggcttcactattaatttccaaaattatacctg

SEQ ID NO: 121 - DNA, 67 bp, synthetic construct
  source 1..67: mol_type = other DNA
agcgccacctggttcttgattcataatagtgaagccacagatgtattatgaatcaagaaccaggtga

SEQ ID NO: 122 - DNA, 67 bp, synthetic construct
  source 1..67: mol_type = other DNA
ggcatcacctggttcttgattcataatacatctgtggcttcactattatgaatcaagaaccaggtgg

SEQ ID NO: 123 - DNA, 67 bp, synthetic construct
  source 1..67: mol_type = other DNA
agcgcaccttctatttttaaactatatagtgaagccacagatgtatatagtttaaaaatagaaggta

SEQ ID NO: 124 - DNA, 67 bp, synthetic construct
  source 1..67: mol_type = other DNA
ggcataccttctatttttaaactatatacatctgtggcttcactatatagtttaaaaatagaaggtg

SEQ ID NO: 125 - DNA, 67 bp, synthetic construct
  source 1..67: mol_type = other DNA
agcgccctgtggtttcttctaatctatagtgaagccacagatgtatagattagaagaaaccacagga

SEQ ID NO: 126 - DNA, 67 bp, synthetic construct
  source 1..67: mol_type = other DNA
ggcatcctgtggtttcttctaatctatacatctgtggcttcactatagattagaagaaaccacaggg

SEQ ID NO: 127 - DNA, 67 bp, synthetic construct
  source 1..67: mol_type = other DNA
agcgccaggatcatgagtttgaattatagtgaagccacagatgtataattcaaactcatgatcctgt

SEQ ID NO: 128 - DNA, 67 bp, synthetic construct
  source 1..67: mol_type = other DNA
ggcaacaggatcatgagtttgaattatacatctgtggcttcactataattcaaactcatgatcctgg

SEQ ID NO: 129 - DNA, 67 bp, synthetic construct
  source 1..67: mol_type = other DNA
agcgcccccagaaattgttaattttatagtgaagccacagatgtataaaattaacaatttctgggga

SEQ ID NO: 130 - DNA, 67 bp, synthetic construct
  source 1..67: mol_type = other DNA
ggcatccccagaaattgttaattttatacatctgtggcttcactataaaattaacaatttctggggg

SEQ ID NO: 131 - DNA, 67 bp, synthetic construct
  source 1..67: mol_type = other DNA
agcgactgtggtttcttctaatctaatagtgaagccacagatgtattagattagaagaaaccacagg

SEQ ID NO: 132 - DNA, 67 bp, synthetic construct
  source 1..67: mol_type = other DNA
ggcacctgtggtttcttctaatctaatacatctgtggcttcactattagattagaagaaaccacagt

SEQ ID NO: 133 - DNA, 67 bp, synthetic construct
  source 1..67: mol_type = other DNA
agcgatgtatgcaaattgatttactatagtgaagccacagatgtatagtaaatcaatttgcatacac

SEQ ID NO: 134 - DNA, 67 bp, synthetic construct
  source 1..67: mol_type = other DNA
ggcagtgtatgcaaattgatttactatacatctgtggcttcactatagtaaatcaatttgcatacat

SEQ ID NO: 135 - DNA, 67 bp, synthetic construct
  source 1..67: mol_type = other DNA
agcgcaccaggtatatgtaatttgaatagtgaagccacagatgtattcaaattacatatacctggta

SEQ ID NO: 136 - DNA, 67 bp, synthetic construct
  source 1..67: mol_type = other DNA
ggcataccaggtatatgtaatttgaatacatctgtggcttcactattcaaattacatatacctggtg

SEQ ID NO: 137 - DNA, 67 bp, synthetic construct
  source 1..67: mol_type = other DNA
agcgccaagatattgtttcaatagattagtgaagccacagatgtaatctattgaaacaatatcttga

SEQ ID NO: 138 - DNA, 67 bp, synthetic construct
  source 1..67: mol_type = other DNA
ggcatcaagatattgtttcaatagattacatctgtggcttcactaatctattgaaacaatatcttgg

SEQ ID NO: 139 - DNA, 67 bp, synthetic construct
  source 1..67: mol_type = other DNA
agcgccgagtcgataatgacaatgaatagtgaagccacagatgtattcattgtcattatcgactcga

SEQ ID NO: 140 - DNA, 67 bp, synthetic construct
  source 1..67: mol_type = other DNA
ggcatcgagtcgataatgacaatgaatacatctgtggcttcactattcattgtcattatcgactcgg

SEQ ID NO: 141 - DNA, 67 bp, synthetic construct
  source 1..67: mol_type = other DNA
agcgatgtgataaatttgttgatgtatagtgaagccacagatgtatacatcaacaaatttatcacac

SEQ ID NO: 142 - DNA, 67 bp, synthetic construct
  source 1..67: mol_type = other DNA
ggcagtgtgataaatttgttgatgtatacatctgtggcttcactatacatcaacaaatttatcacat

SEQ ID NO: 143 - DNA, 67 bp, synthetic construct
  source 1..67: mol_type = other DNA
agcgcgactgtattagatcattaatatagtgaagccacagatgtatattaatgatctaatacagtca

SEQ ID NO: 144 - DNA, 67 bp, synthetic construct
  source 1..67: mol_type = other DNA
ggcatgactgtattagatcattaatatacatctgtggcttcactatattaatgatctaatacagtcg

SEQ ID NO: 145 - DNA, 67 bp, synthetic construct
  source 1..67: mol_type = other DNA
agcgccctgactgtattagatcattatagtgaagccacagatgtataatgatctaatacagtcagga

SEQ ID NO: 146 - DNA, 67 bp, synthetic construct
  source 1..67: mol_type = other DNA
ggcatcctgactgtattagatcattatacatctgtggcttcactataatgatctaatacagtcaggg

SEQ ID NO: 147 - DNA, 67 bp, synthetic construct
  source 1..67: mol_type = other DNA
agcgatatgatgaagactattgataatagtgaagccacagatgtattatcaatagtcttcatcatag

SEQ ID NO: 148 - DNA, 67 bp, synthetic construct
  source 1..67: mol_type = other DNA
ggcactatgatgaagactattgataatacatctgtggcttcactattatcaatagtcttcatcatat

SEQ ID NO: 149 - DNA, 67 bp, synthetic construct
  source 1..67: mol_type = other DNA
agcgcccactcgatttctcttttgaatagtgaagccacagatgtattcaaaagagaaatcgagtgga

SEQ ID NO: 150 - DNA, 67 bp, synthetic construct
  source 1..67: mol_type = other DNA
ggcatccactcgatttctcttttgaatacatctgtggcttcactattcaaaagagaaatcgagtggg

SEQ ID NO: 151 - DNA, 67 bp, synthetic construct
  source 1..67: mol_type = other DNA
agcgccaagtgcaacagaattgtttatagtgaagccacagatgtataaacaattctgttgcacttga

SEQ ID NO: 152 - DNA, 67 bp, synthetic construct
  source 1..67: mol_type = other DNA
ggcatcaagtgcaacagaattgtttatacatctgtggcttcactataaacaattctgttgcacttgg

SEQ ID NO: 153 - DNA, 67 bp, synthetic construct
  source 1..67: mol_type = other DNA
agcgccacatccttctgtaatcttaatagtgaagccacagatgtattaagattacagaaggatgtga

SEQ ID NO: 154 - DNA, 67 bp, synthetic construct
  source 1..67: mol_type = other DNA
ggcatcacatccttctgtaatcttaatacatctgtggcttcactattaagattacagaaggatgtgg

SEQ ID NO: 155 - DNA, 67 bp, synthetic construct
  source 1..67: mol_type = other DNA
agcgacacgatttctttgttgacatatagtgaagccacagatgtatatgtcaacaaagaaatcgtgc

SEQ ID NO: 156 - DNA, 67 bp, synthetic construct
  source 1..67: mol_type = other DNA
ggcagcacgatttctttgttgacatatacatctgtggcttcactatatgtcaacaaagaaatcgtgt

SEQ ID NO: 157 - DNA, 67 bp, synthetic construct
  source 1..67: mol_type = other DNA
agcgcgggtacagttctggttttatatagtgaagccacagatgtatataaaaccagaactgtaccca

SEQ ID NO: 158 - DNA, 67 bp, synthetic construct
  source 1..67: mol_type = other DNA
ggcatgggtacagttctggttttatatacatctgtggcttcactatataaaaccagaactgtacccg

SEQ ID NO: 159 - DNA, 67 bp, synthetic construct
  source 1..67: mol_type = other DNA
agcgagaggagatattagttgatttatagtgaagccacagatgtataaatcaactaatatctcctcg

SEQ ID NO: 160 - DNA, 67 bp, synthetic construct
  source 1..67: mol_type = other DNA
ggcacgaggagatattagttgatttatacatctgtggcttcactataaatcaactaatatctcctct

SEQ ID NO: 161 - DNA, 67 bp, synthetic construct
  source 1..67: mol_type = other DNA
agcgctcctactatttttcattagtatagtgaagccacagatgtatactaatgaaaaatagtaggat

SEQ ID NO: 162 - DNA, 67 bp, synthetic construct
  source 1..67: mol_type = other DNA
ggcaatcctactatttttcattagtatacatctgtggcttcactatactaatgaaaaatagtaggag

SEQ ID NO: 163 - DNA, 67 bp, synthetic construct
  source 1..67: mol_type = other DNA
agcgccagtatctcttgatttcttaatagtgaagccacagatgtattaagaaatcaagagatactga

SEQ ID NO: 164 - DNA, 67 bp, synthetic construct
  source 1..67: mol_type = other DNA
ggcatcagtatctcttgatttcttaatacatctgtggcttcactattaagaaatcaagagatactgg

SEQ ID NO: 165 - DNA, 67 bp, synthetic construct
  source 1..67: mol_type = other DNA
agcgccggattgattcttttgtatgatagtgaagccacagatgtatcatacaaaagaatcaatccga

SEQ ID NO: 166 - DNA, 67 bp, synthetic construct
  source 1..67: mol_type = other DNA
ggcatcggattgattcttttgtatgatacatctgtggcttcactatcatacaaaagaatcaatccgg

SEQ ID NO: 167 - DNA, 67 bp, synthetic construct
  source 1..67: mol_type = other DNA
agcgacagtatctacattgtttagtatagtgaagccacagatgtatactaaacaatgtagatactgc

SEQ ID NO: 168 - DNA, 67 bp, synthetic construct
  source 1..67: mol_type = other DNA
ggcagcagtatctacattgtttagtatacatctgtggcttcactatactaaacaatgtagatactgt

SEQ ID NO: 169 - RNA, 27 nt, synthetic construct
  source 1..27: mol_type = other RNA
attttaattttctaatagatcgttgtc

SEQ ID NO: 170 - RNA, 25 nt, synthetic construct
  source 1..25: mol_type = other RNA
caacgatctattagaaaattaaaat

SEQ ID NO: 171 - RNA, 27 nt, synthetic construct
  source 1..27: mol_type = other RNA
tatatatatagatcttgttacctagta

SEQ ID NO: 172 - RNA, 25 nt, synthetic construct
  source 1..25: mol_type = other RNA
ctaggtaacaagatctatatatata

SEQ ID NO: 173 - RNA, 27 nt, synthetic construct
  source 1..27: mol_type = other RNA
atatctaatgatctatagatctgtcat

SEQ ID NO: 174 - RNA, 25 nt, synthetic construct
  source 1..25: mol_type = other RNA
gacagatctatagatcattagatat

SEQ ID NO: 175 - RNA, 27 nt, synthetic construct
  source 1..27: mol_type = other RNA
ttaacatttcattttgtatctgtatta

SEQ ID NO: 176 - RNA, 25 nt, synthetic construct
  source 1..25: mol_type = other RNA
atacagatacaaaatgaaatgttaa

SEQ ID NO: 177 - RNA, 27 nt, synthetic construct
  source 1..27: mol_type = other RNA
tgacttaggaattttgaacaaggttat

SEQ ID NO: 178 - RNA, 25 nt, synthetic construct
  source 1..25: mol_type = other RNA
aaccttgttcaaaattcctaagtca

SEQ ID NO: 179 - DNA, 4506 bp, synthetic construct
  source 1..4506: mol_type = other DNA
ttaatgtagtcttatgcaatactcttgtagtcttgcaacatggtaacgatgagttagcaacatgccttacaaggagagaaaaagcaccgtgcatgccgattggtggaagtaaggtggtacgatcgtgccttattaggaaggcaacagacgggtctgacatggattggacgaaccactgaattgccgcattgcagagatattgtatttaagtgcctagctcgatacataaacgggtctctctggttagaccagatctgagcctgggagctctctggctaactagggaacccactgcttaagcctcaataaagcttgccttgagtgcttcaagtagtgtgtgcccgtctgttgtgtgactctggtaactagagatccctcagacccttttagtcagtgtggaaaatctctagcagtggcgcccgaacagggacttgaaagcgaaagggaaaccagaggagctctctcgacgcaggactcggcttgctgaagcgcgcacggcaagaggcgaggggcggcgactggtgagtacgccaaaaattttgactagcggaggctagaaggagagagatgggtgcgagagcgtcagtattaagcgggggagaattagatcgcgatgggaaaaaattcggttaaggccagggggaaagaaaaaatataaattaaaacatatagtatgggcaagcagggagctagaacgattcgcagttaatcctggcctgttagaaacatcagaaggctgtagacaaatactgggacagctacaaccatcccttcagacaggatcagaagaacttagatcattatataatacagtagcaaccctctattgtgtgcatcaaaggatagagataaaagacaccaaggaagctttagacaagatagaggaagagcaaaacaaaagtaagaccaccgcacagcaagcggccgctgatcttcagacctggaggaggagatatgagggacaattggagaagtgaattatataaatataaagtagtaaaaattgaaccattaggagtagcacccaccaaggcaaagagaagagtggtgcagagagaaaaaagagcagtgggaataggagctttgttccttgggttcttgggagcagcaggaagcactatgggcgcagcgtcaatgacgctgacggtacaggccagacaattattgtctggtatagtgcagcagcagaacaatttgctgagggctattgaggcgcaacagcatctgttgcaactcacagtctggggcatcaagcagctccaggcaagaatcctggctgtggaaagatacctaaaggatcaacagctcctggggatttggggttgctctggaaaactcatttgcaccactgctgtgccttggaatgctagttggagtaataaatctctggaacagatttggaatcacacgacctggatggagtgggacagagaaattaacaattacacaagcttaatacactccttaattgaagaatcgcaaaaccagcaagaaaagaatgaacaagaattattggaattagataaatgggcaagtttgtggaattggtttaacataacaaattggctgtggtatataaaattattcataatgatagtaggaggcttggtaggtttaagaatagtttttgctgtactttctatagtgaatagagttaggcagggatattcaccattatcgtttcagacccacctcccaaccccgaggggacaattctagatcttgagacaaatggcagtattcatccacaattttaaaagaaaaggggggattggggggtacagtgcaggggaaagaatagtagacataatagcaacagacatacaaactaaagaattacaaaaacaaattacaaaaattcaaaattttcgggtttattacagggacagcagagatccactttggcgccggctcgagcgagctgcagtaacgccattttgcaaggcatggaaaaataccaaaccaagaatagagaagttcagatcaagggcgggtacatgaaaatagctaacgttgggccaaacaggatatctgcggtgagcagtttcggccccggcccggggccaagaacagatggtcaccgcagtttcggccccggcccgaggccaagaacagatggtccccagatatggcccaaccctcagcagtttcttaagacccatcagatgtttccaggctcccccaaggacctgaaatgaccctgcgccttatttgaattaaccaatcagcctgcttctcgcttctgttcgcgcgcttctgcttcccgagctctataaaagagctcacaacccctcactcggcgcgccagtcctccgacagactgagtcggatccgccaccatggtgagcaagggcgaggaggataacatggccatcatcaaggagttcatgcgcttcaaggtgcacatggagggctccgtgaacggccacgagttcgagatcgagggcgagggcgagggccgcccctacgagggcacccagaccgccaagctgaaggtgaccaagggtggccccctgcccttcgcctgggacatcctgtcccctcagttcatgtacggctccaaggcctacgtgaagcaccccgccgacatccccgactacttgaagctgtccttccccgagggcttcaagtgggagcgcgtgatgaacttcgaggacggcggcgtggtgaccgtgacccaggactcctccctgcaggacggcgagttcatctacaaggtgaagctgcgcggcaccaacttcccctccgacggccccgtaatgcagaaaaagacaatgggctgggaggcctcctccgagcggatgtaccccgaggacggcgccctgaagggcgagatcaagcagaggctgaagctgaaggacggcggccactacgacgctgaggtcaagaccacctacaaggccaagaagcccgtgcagctgcccggcgcctacaacgtcaacatcaagttggacatcacctcccacaacgaggactacaccatcgtggaacagtacgaacgcgccgagggccgccactccaccggcggcatggacgagctgtacaagtgagcggccgcatattgctgtttgaatgaggcttcagtactttacagaatcgttgcctgcacatcttggaaacacttgctgggattacttcttcaggttaacccaacagaaggctaaagaaggtatattgctgttgacagtgagcgaaacgatctattagaaaattaatagtgaagccacagatgtattaattttctaatagatcgttgtgcctactgcctcggacttcaaggggctactttaggagcaattatcttgtttactaaaactgaataccttgctatctctttgatacatttttacaaagctgaattaaaatggtataaattaaatcacttttttacgcgttaagtcgacaatcaacctctggattacaaaatttgtgaaagattgactggtattcttaactatgttgctccttttacgctatgtggatacgctgctttaatgcctttgtatcatgctattgcttcccgtatggctttcattttctcctccttgtataaatcctggttgctgtctctttatgaggagttgtggcccgttgtcaggcaacgtggcgtggtgtgcactgtgtttgctgacgcaacccccactggttggggcattgccaccacctgtcagctcctttccgggactttcgctttccccctccctattgccacggcggaactcatcgccgcctgccttgcccgctgctggacaggggctcggctgttgggcactgacaattccgtggtgttgtcggggaaatcatcgtcctttccttggctgctcgcctgtgttgccacctggattctgcgcgggacgtccttctgctacgtcccttcggccctcaatccagcggaccttccttcccgcggcctgctgccggctctgcggcctcttccgcgtcttcgccttcgccctcagacgagtcggatctccctttgggccgcctccccgcgtcgactttaagaccaatgacttacaaggcagctgtagatcttagccactttttaaaagaaaaggggggactggaagggctaattcactcccaacgaagacaagatctgctttttgcttgtactgggtctctctggttagaccagatctgagcctgggagctctctggctaactagggaacccactgcttaagcctcaataaagcttgccttgagtgcttcaagtagtgtgtgcccgtctgttgtgtgactctggtaactagagatccctcagacccttttagtcagtgtggaaaatctctagcagtacgtatagtagttcatgtcatcttattattcagtatttataacttgcaaagaaatgaatatcagagagtgagaggaacttgtttattgcagcttataatggttacaaataaagcaatagcatcacaaatttcacaaataaagcatttttttcactgcattctagttgtggtttgtccaaactcatcaatgtatcttatcatgtctg

SEQ ID NO: 180 - protein, 512 aa, Maraba virus
MLRLFLFCFLALGAHSKFTIVFPHHQKGNWKNVPSTYHYCPSSSDQNWHNDLTGVSLHVKIPKSHKAIQADGWMCHAAKWVTTCDFRWYGPKYITHSIHSMSPTLEQCKTSIEQTKQGVWINPGFPPQSCGYATVTDAEVVVVQATPHHVLVDEYTGEWIDSQLVGGKCSKEVCQTVHNSTVWHADYKITGLCESNLASVDITFFSEDGQKTSLGKPNTGFRSNHFAYESGEKACRMQYCTQWGIRLPSGVWFELVDKDLFQAAKLPECPRGSSISAPSQTSVDVSLIQDVERILDYSLCQETWSKIRAKLPVSPVDLSYLAPKNPGSGPAFTIINGTLKYFETRYIRVDISNPIIPHMVGTMSGTTTERELWNDWYPYEDVEIGPNGVLKTPTGFKFPLYMIGHGMLDSDLHKSSQAQVFEHPHAKDAASQLPDDETLFFGDTGLSKNPVELVEGWFSSWKSTLASFFLIIGLGVALIFIIRIIVAIRYKYKGRKTQKIYNDVEMSRLGNK

SEQ ID NO: 181 - DNA, 1539 bp, Maraba virus
  source 1..1539: mol_type = other DNA
atgttgagactttttctcttttgtttcttggccttaggagcccactccaaatttactatagtattccctcatcatcaaaaagggaattggaagaatgtgccttccacatatcattattgcccttctagttctgaccagaattggcataatgatttgactggagttagtcttcatgtgaaaattcccaaaagtcacaaagctatacaagcagatggctggatgtgccacgctgctaaatgggtgactacttgtgacttcagatggtacggacccaaatacatcacgcattccatacactctatgtcacccaccctagaacagtgcaagaccagtattgagcagacaaagcaaggagtttggattaatccaggctttccccctcaaagctgcggatatgctacagtgacggatgcagaggtggttgttgtacaagcaacacctcatcatgtgttggttgatgagtacacaggagaatggattgactcacaattggtggggggcaaatgttccaaggaggtttgtcaaacggttcacaactcgaccgtgtggcatgctgattacaagattacagggctgtgcgagtcaaatctggcatcagtggatatcaccttcttctctgaggatggtcaaaagacgtctttgggaaaaccgaacactggattcaggagtaatcactttgcttacgaaagtggagagaaggcatgccgtatgcagtactgcacacaatgggggatccgactaccttctggagtatggtttgaattagtggacaaagatctcttccaggcggcaaaattgcctgaatgtcctagaggatccagtatctcagctccttctcagacttctgtggatgttagtttgatacaagacgtagagaggatcttagattactctctatgccaggagacgtggagtaagatacgagccaagcttcctgtatctccagtagatctgagttatctcgccccaaaaaatccagggagcggaccggccttcactatcattaatggcactttgaaatatttcgaaacaagatacatcagagttgacataagtaatcccatcatccctcacatggtgggaacaatgagtggaaccacgactgagcgtgaattgtggaatgattggtatccatatgaagacgtagagattggtccaaatggggtgttgaaaactcccactggtttcaagtttccgctgtacatgattgggcacggaatgttggattccgatctccacaaatcctcccaggctcaagtcttcgaacatccacacgcaaaggacgctgcatcacagcttcctgatgatgagactttattttttggtgacacaggactatcaaaaaacccagtagagttagtagaaggctggttcagtagctggaagagcacattggcatcgttctttctgattataggcttgggggttgcattaatcttcatcattcgaattattgttgcgattcgctataaatacaaggggaggaagacccaaaaaatttacaatgatgtcgagatgagtcgattgggaaataaataa

SEQ ID NO: 182 - protein, 511 aa, Vesicular stomatitis virus
MKCLLYLAFLFIGVNCKFTIVFPHNQKGNWKNVPSNYHYCPSSSDLNWHNDLIGTALQVKMPKSHKAIQADGWMCHASKWVTTCDFRWYGPKYITHSIRSFTPSVEQCKESIEQTKQGTWLNPGFPPQSCGYATVTDAEAVIVQVTPHHVLVDEYTGEWVDSQFINGKCSNYICPTVHNSTTWHSDYKVKGLCDSNLISMDITFFSEDGELSSLGKEGTGFRSNYFAYETGGKACKMQYCKHWGVRLPSGVWFEMADKDLFAAARFPECPEGSSISAPSQTSVDVSLIQDVERILDYSLCQETWSKIRAGLPISPVDLSYLAPKNPGTGPAFTIINGTLKYFETRYIRVDIAAPILSRMVGMISGTTTERELWDDWAPYEDVEIGPNGVLRTSSGYKFPLYMIGHGMLDSDLHLSSKAQVFEHPHIQDAASQLPDDESLFFGDTGLSKNPIELVEGWFSSWKSSIASFFFIIGLIIGLFLVLRVGIHLCIKLKHTKKRQIYTDIEMNRLGK

SEQ ID NO: 183 - DNA, 1536 bp, Vesicular stomatitis virus
  source 1..1536: mol_type = other DNA
atgaagtgccttttgtacttagcctttttattcattggggtgaattgcaagttcaccatagtttttccacacaaccaaaaaggaaactggaaaaatgttccttctaattaccattattgcccgtcaagctcagatttaaattggcataatgacttaataggcacagccttacaagtcaaaatgcccaagagtcacaaggctattcaagcagacggttggatgtgtcatgcttccaaatgggtcactacttgtgatttccgctggtatggaccgaagtatataacacattccatccgatccttcactccatctgtagaacaatgcaaggaaagcattgaacaaacgaaacaaggaacttggctgaatccaggcttccctcctcaaagttgtggatatgcaactgtgacggatgccgaagcagtgattgtccaggtgactcctcaccatgtgctggttgatgaatacacaggagaatgggttgattcacagttcatcaacggaaaatgcagcaattacatatgccccactgtccataactctacaacctggcattctgactataaggtcaaagggctatgtgattctaacctcatttccatggacatcaccttcttctcagaggacggagagctatcatccctgggaaaggagggcacagggttcagaagtaactactttgcttatgaaactggaggcaaggcctgcaaaatgcaatactgcaagcattggggagtcagactcccatcaggtgtctggttcgagatggctgataaggatctctttgctgcagccagattccctgaatgcccagaagggtcaagtatctctgctccatctcagacctcagtggatgtaagtctaattcaggacgttgagaggatcttggattattccctctgccaagaaacctggagcaaaatcagagcgggtcttccaatctctccagtggatctcagctatcttgctcctaaaaacccaggaaccggtcctgctttcaccataatcaatggtaccctaaaatactttgagaccagatacatcagagtcgatattgctgctccaatcctctcaagaatggtcggaatgatcagtggaactaccacagaaagggaactgtgggatgactgggcaccatatgaagacgtggaaattggacccaatggagttctgaggaccagttcaggatataagtttcctttatacatgattggacatggtatgttggactccgatcttcatcttagctcaaaggctcaggtgttcgaacatcctcacattcaagacgctgcttcgcaacttcctgatgatgagagtttattttttggtgatactgggctatccaaaaatccaatcgagcttgtagaaggttggttcagtagttggaaaagctctattgcctcttttttctttatcatagggttaatcattggactattcttggttctccgagttggtatccatctttgcattaaattaaagcacaccaagaaaagacagatttatacagacatagagatgaaccgacttggaaagtaa

SEQ ID NO: 184 - protein, 517 aa, Vesicular stomatitis virus
MLSYLIFALAVSPILGKIEIVFPQHTTGDWKRVPHEYNYCPTSADKNSHGTQTGIPVELTMPKGLTTHQVEGFMCHSALWMTTCDFRWYGPKYITHSIHNEEPTDYQCLEAIKSYKDGVSFNPGFPPQSCGYGTVTDAEAHIVTVTPHSVKVDEYTGEWIDPHFIGGRCKGQICETVHNSTKWFTSSDGESVCSQLFTLVGGIFFSDSEEITSMGLPETGIRSNYFPYISTEGICKMPFCRKQGYKLKNDLWFQIMDPDLDKTVRDLPHIKDCDLSSSIITPGEHATDISLISDVERILDYALCQNTWSKIESGEPITPVDLSYLGPKNPGVGPVFTIINGSLHYFTSKYLRVELESPVIPRMEGKVAGTRIVRQLWDQWFPFGEVEIGPNGVLKTKQGYKFPLHIIGTGEVDSDIKMERVVKHWEHPHIEAAQTFLKKDDTGEVLYYGDTGVSKNPVELVEGWFSGWRSSLMGVLAVIIGFVILMFLIKLIGVLSSLFRPKRRPIYKSDVEMAHFR

SEQ ID NO: 185 - DNA, 1554 bp, Vesicular stomatitis virus
  source 1..1554: mol_type = other DNA
atgttgtcttatctaatctttgcacttgccgtttcgcccattttgggcaaaattgaaattgtgtttcctcaacataccactggggattggaagagagttccccatgaatataattattgccctaccagcgcagacaagaactcacatgggactcaaacaggaatccctgttgagttaacaatgccaaaaggactaacaacccatcaagttgaaggatttatgtgtcactcagccttgtggatgaccacttgtgacttcagatggtatgggccaaaatacataacccattccatacataatgaagagcctacagattatcaatgtttggaggccattaagtcatacaaagatggagtcagtttcaatccagggtttcctcctcagagctgcgggtatggcacagttaccgatgccgaagcccatattgtgacagttactccccactctgtcaaagtggacgagtacacgggggaatggatcgatccacatttcatcggaggaaggtgcaaaggacaaatttgtgaaacagtccataattccacaaaatggtttacgtcctctgatggagaaagtgtctgcagtcaattgtttactttggttggaggaatttttttctctgattcagaagagattacctccatggggttaccagaaacaggaatcagaagtaattacttcccctacatatctacagagggaatttgcaaaatgccgttttgcagaaaacaggggtacaagcttaaaaatgacctctggttccagatcatggacccagacctggataaaacggttagagatctccctcatattaaggactgtgacctctcctcgtccataatcacaccaggagaacatgctacagacatctcactgatatcagatgttgaaaggatcctggactatgctctttgtcagaatacatggagtaaaattgaatcgggagaaccaattactccggtagatctcagctatcttgggccaaaaaacccaggggttgggccggtcttcaccatcattaacggttccctgcattattttacatcgaagtatctgcgagtcgaattagaaagtcctgtcatacccagaatggaaggaaaagttgcaggaactaggattgtacggcaattgtgggatcagtggtttcctttcggagaagttgagattggacccaatggtgtgttgaaaacgaagcaagggtataaattcccactacacatcattggaactggagaagtagacagtgacatcaaaatggaaagggttgtcaagcactgggaacacccccatattgaggccgctcagacatttttaaaaaaagatgacacaggagaagtcctttattatggcgacaccggagtgtcgaaaaatccagttgaattagtcgagggatggtttagtggatggaggagctccctcatgggagtgctggctgtgattataggatttgtgattttaatgtttttaattaaattgattggagtcttatctagccttttcagacctaaacgcaggccaatctacaaatcagacgtggaaatggctcatttccgttaa

SEQ ID NO: 186 - protein, 511 aa, synthetic construct
MKCLLYLAFLFIGVNCKFTIVFPHNQKGNWKNVPSNYHYCPSSSDLNWHNDLIGTALQVKMPKSHKAIQADGWMCHASKWVTTCDFRWYGPKYITHSIRSFTPSVEQCKESIEQTKQGTWLNPGFPPQSCGYATVTDAEAVIVQVTPHHVLVDEYTGEWVDSQFINGKCSNYICPTVHNSTTWHSDYKVKGLCDSNLISMDITFFSEDGELSSLGKEGTGFRSNYFAYENGGKACKMQYCKHWGVRLPSGVWFEMADKDLFAAARFPECPEGSSISAPSQTSVDVSLIQDVERILDYSLCQETWSKIRAGLPISPVDLSYLAPKNPGTGPAFTIINGTLKYFETRYIRVDIAAPILSRMVGMISGTTAERELWDDWAPYEDVEIGPNGVLRTSSGYKFPLYMIGHGMLDSDLHLSSKAQVFEHPHIQDAASQLPDDESLFFGDTGLSKNPIELVEGWFSSWKSSIASFFFIIGLIIGLFLVLRVGIHLCIKLKHTKKRQIYTDIEMNRLGK

SEQ ID NO: 187 - DNA, 1536 bp, synthetic construct
  source 1..1536: mol_type = other DNA
atgaagtgccttttgtacttagcctttttattcattggggtgaattgcaagttcaccatagtttttccacacaaccaaaaaggaaactggaaaaatgttccttctaattaccattattgcccgtcaagctcagatttaaattggcataatgacttaataggcacagccttacaagtcaaaatgcccaagagtcacaaggctattcaagcagacggttggatgtgtcatgcttccaaatgggtcactacttgtgatttccgctggtatggaccgaagtatataacacattccatccgatccttcactccatctgtagaacaatgcaaggaaagcattgaacaaacgaaacaaggaacttggctgaatccaggcttccctcctcaaagttgtggatatgcaactgtgacggatgccgaagcagtgattgtccaggtgactcctcaccatgtgctggttgatgaatacacaggagaatgggttgattcacagttcatcaacggaaaatgcagcaattacatatgccccactgtccataactctacaacctggcattctgactataaggtcaaagggctatgtgattctaacctcatttccatggacatcaccttcttctcagaggacggagagctatcatccctgggaaaggagggcacagggttcagaagtaactactttgcttatgaaaatggaggcaaggcctgcaaaatgcaatactgcaagcattggggagtcagactcccatcaggtgtctggttcgagatggctgataaggatctctttgctgcagccagattccctgaatgcccagaagggtcaagtatctctgctccatctcagacctcagtggatgtaagtctaattcaggacgttgagaggatcttggattattccctctgccaagaaacctggagcaaaatcagagcgggtcttccaatctctccagtggatctcagctatcttgctcctaaaaacccaggaaccggtcctgctttcaccataatcaatggtaccctaaaatactttgagaccagatacatcagagtcgatattgctgctccaatcctctcaagaatggtcggaatgatcagtggaactaccgcagaaagggaactgtgggatgactgggcaccatatgaagacgtggaaattggacccaatggagttctgaggaccagttcaggatataagtttcctttatacatgattggacatggtatgttggactccgatcttcatcttagctcaaaggctcaggtgttcgaacatcctcacattcaagacgctgcttcgcaacttcctgatgatgagagtttattttttggtgatactgggctatccaaaaatccaatcgagcttgtagaaggttggttcagtagttggaaaagctctattgcctcttttttctttatcatagggttaatcattggactattcttggttctccgagttggtatccatctttgcattaaattaaagcacaccaagaaaagacagatttatacagacatagagatgaaccgacttggaaagtaa

SEQ ID NO: 188 - protein, 512 aa, Cocal virus
MNFLLLTFIVLPLCSHAKFSIVFPQSQKGNWKNVPSSYHYCPSSSDQNWHNDLLGITMKVKMPKTHKAIQADGWMCHAAKWITTCDFRWYGPKYITHSIHSIQPTSEQCKESIKQTKQGTWMSPGFPPQNCGYATVTDSVAVVVQATPHHVLVDEYTGEWIDSQFPNGKCETEECETVHNSTVWYSDYKVTGLCDATLVDTEITFFSEDGKKESIGKPNTGYRSNYFAYEKGDKVCKMNYCKHAGVRLPSGVWFEFVDQDVYAAAKLPECPVGATISAPTQTSVDVSLILDVERILDYSLCQETWSKIRSKQPVSPVDLSYLAPKNPGTGPAFTIINGTLKYFETRYIRIDIDNPIISKMVGKISGSQTERELWTEWFPYEGVEIGPNGILKTPTGYKFPLFMIGHGMLDSDLHKTSQAEVFEHPHLAEAPKQLPEEETLFFGDTGISKNPVELIEGWFSSWKSTVVTFFFAIGVFILLYVVARIVIAVRYRYQGSNNKRIYNDIEMSRFRK

SEQ ID NO: 189 - DNA, 1539 bp, Cocal virus
  source 1..1539: mol_type = other DNA
atgaatttcctactcttgacatttattgtgttgccgttgtgcagccacgccaagttctccattgtattccctcaaagccaaaaaggcaattggaagaatgtaccatcatcttaccattactgcccttcaagttcggatcaaaactggcacaatgatttgcttggaatcacaatgaaagtcaaaatgcccaaaacacacaaagctattcaagcagacgggtggatgtgtcatgctgccaaatggatcactacctgtgactttcgctggtacggacccaaatacatcactcactccattcattccatccagcctacttcagagcagtgtaaagaaagcatcaagcaaacaaaacaaggtacttggatgagtcctggcttccctccacagaactgcgggtatgcaacagtaacagactctgtcgctgttgtcgtccaagccactcctcatcatgtcttggttgatgaatatactggagaatggatcgactctcaattccccaacgggaaatgtgaaaccgaagagtgcgagaccgtccacaactctaccgtatggtactctgactacaaagtaactggattatgtgacgcaactctggtagacacagagatcaccttcttctctgaagatggcaaaaaagaatctatcgggaagcccaacacaggctataggagcaactacttcgcttatgagaaaggggacaaagtatgtaaaatgaactactgcaagcatgcgggtgtgaggttgccttccggggtttggtttgagtttgtggatcaggatgtctacgccgccgccaaacttccagaatgccccgttggtgccactatctccgctccgacacagacctctgttgacgtaagtctcattctagatgtagagagaattttagattactctctgtgtcaagagacatggagcaagatccggtccaaacagccagtatcccctgttgaccttagttacttggcccccaagaatcctgggaccggaccggcattcacaatcatcaatggcactctgaagtactttgagaccagatacattcggattgatatagacaatccaatcatctccaagatggtggggaaaataagtggcagtcaaacagaacgagaattgtggacagagtggttcccctacgagggtgtcgagatagggccaaatgggattctcaaaacccctacaggatacaaattcccactcttcatgataggacacgggatgctagattccgacttgcacaagacgtcccaagcagaggtctttgaacatcctcaccttgcagaagcaccaaagcagttgccggaggaggagactttattttttggtgacacaggaatctccaaaaatccggtcgaactgattgaagggtggtttagtagttggaagagcactgtagtcacctttttctttgccataggagtatttatactactgtatgtagtggccagaattgtgatcgcagtgagatacagatatcaaggctcaaataacaaaagaatttacaatgatattgagatgagcagatttagaaaatga

SEQ ID NO: 190 - protein, 529 aa, Piry virus
MDLFPILVVVLMTDTVLGKFQIVFPDQNELEWRPVVGDSRHCPQSSEMQFDGSRSQTILTGKAPVGITPSKSDGFICHAAKWVTTCDFRWYGPKYITHSIHHLRPTTSDCETALQRYKDGSLINLGFPPESCGYATVTDSEAMLVQVTPHHVGVDDYRGHWIDPLFPGGECSTNFCDTVHNSSVWIPKSQKTDICAQSFKNIKMTASYPSEGALVSDRFAFHSAYHPNMPGSTVCIMDFCEQKGLRFTNGEWMGLNVEQSIREKKISAIFPNCVAGTEIRATLESEGARTLTWETQRMLDYSLCQNTWDKVSRKEPLSPLDLSYLSPRAPGKGMAYTVINGTLHSAHAKYIRTWIDYGEMKEIKGGRGEYSKAPELLWSQWFDFGPFKIGPNGLLHTGKTFKFPLYLIGAGIIDEDLHELDEAAPIDHPQMPDAKSVLPEDEEIFFGDTGVSKNPIELIQGWFSNWRESVMAIVGIVLLIVVTFLAIKTVRVLNCLWRPRKKRIVRQEVDVESRLNHFEMRGFPEYVKR

SEQ ID NO: 191 - DNA, 1590 bp, Piry virus
  source 1..1590: mol_type = other DNA
atggatctctttcccattttggtcgtggtgctcatgacagatactgtcttagggaagtttcaaattgtcttcccggatcagaatgaactggagtggagaccagttgtgggtgactctcggcattgcccacagtcatcagaaatgcaattcgatggaagcagatcccagaccatactgactgggaaagctcccgtggggatcacgccctctaaatcagatggatttatctgccatgccgcaaaatgggtgacaacatgtgatttcaggtggtatgggccgaaatacatcactcattcaatacatcatctgagaccgacaacatcagactgtgagacagctctccaaaggtataaagatgggagcttaatcaatcttggattccccccagaatcctgcggttatgcaacagtcacagattctgaggcaatgttggtccaagtgactccccaccacgttggggtggatgattatagaggtcactggatcgacccactatttccaggaggagaatgctccaccaatttttgtgatacagtccacaattcatcggtgtggatccccaagagtcaaaagactgacatctgtgcccagtctttcaaaaatatcaagatgaccgcatcttacccctcagaaggagcattggtgagtgacagatttgccttccacagtgcatatcatccaaatatgccggggtcaactgtttgcataatggacttttgcgaacaaaaggggttgagattcacaaatggagagtggatgggtctcaatgtggagcaatccatccgagagaagaagataagtgccatcttcccaaattgtgttgcagggactgaaatccgagccacactagaatcagaaggggcaagaactttgacgtgggagactcaaagaatgctagattactctttgtgtcagaacacctgggacaaagtttccaggaaagaacctctcagtccgcttgacttgagctatctgtcaccaagggctccagggaaaggcatggcctataccgtcataaacggaaccctgcattcggctcatgctaaatacattagaacctggattgattatggagaaatgaaggaaattaaaggtggacgtggagaatattccaaggctcctgagctcctctggtcccagtggttcgattttggaccgttcaaaattggaccgaatggactcctgcacacagggaaaacctttaaattccctctttatttgatcggagcaggcataattgacgaagatctgcatgaactagatgaggctgctcccattgatcacccacaaatgcctgacgcgaaaagcgttcttccagaagatgaagagatattcttcggagacacaggtgtatccaaaaaccctatcgagttgattcaaggatggttctcaaattggagagagagtgtaatggcaatagtcggaattgttctactcatcgttgtgacatttctggcgatcaagacggtccgggtgcttaattgtctctggagacccagaaagaaaagaatcgtcagacaagaagtagatgttgaatcccgactaaaccattttgagatgagaggctttcctgaatatgttaagagataa

SEQ ID NO: 192 - protein, 563 aa, Influenza virus
MNTQILVFALVAVIPTNADKICLGHHAVSNGTKVNTLTERGVEVVNATETVERTNIPKICSKGKRTTDLGQCGLLGTITGPPQCDQFLEFSADLIIERREGNDVCYPGKFVNEEALRQILRGSGGIDKETMGFTYSGIRTNGTTSACRRSGSSFYAEMEWLLSNTGNASFPQMTKSYKNTRRESALIVWGIHHSGSTTEQTKLYGSGNKLITVGSSKYHQSFVPSPGTRPQINGQSGRIDFHWLILDPNDTVTFSFNGAFIAPNRASFLRGKSMGIQSDVQVDANCEGECYHSGGTITSRLPFQNINSRAVGKCPRYVKQESLLLATGMKNVPEPSKKRKKRGLFGAIAGFIENGWEGLVDGWYGFRHQNAQGEGTAADYKSTQSAIDQITGKLNRLIEKTNQQFELIDNEFTEVEKQIGNLINWTKDSITEVWSYNAELIVAMENQHTIDLADSEMNRLYERVRKQLRENAEEDGTGCFEIFHKCDDDCMASIRNNIYDHSKYREEAMQNRIQIDPVKLSSGYKDVILWFSFGASCFLLLAIAMGLVFICVKNGNMRCTICI

SEQ ID NO: 193 - DNA, 1692 bp, Influenza virus
  source 1..1692: mol_type = other DNA
atgaacactcaaatcctggttttcgcccttgtggcagtcatccccacaaatgcagacaaaatttgtcttggacatcatgctgtatcaaatggcaccaaagtaaacacactcactgagagaggagtagaagttgtcaatgcaacggaaacagtggagcggacaaacatccccaaaatttgctcaaaagggaaaagaaccactgatcttggccaatgcggactgttagggaccattaccggaccacctcaatgcgaccaatttctagaattttcagctgatctaataatcgagagacgagaaggaaatgatgtttgttacccggggaagtttgttaatgaagaggcattgcgacaaatcctcagaggatcaggtgggattgacaaagaaacaatgggattcacatatagtggaataaggaccaacggaacaactagtgcatgtagaagatcagggtcttcattctatgcagaaatggagtggctcctgtcaaatacaggcaatgcttctttcccacaaatgacaaaatcatacaaaaacacaaggagagaatcagctctgatagtctggggaatccaccattcaggatcaaccaccgaacagaccaaactatatgggagtggaaataaactgataacagtcgggagttccaaatatcatcaatcttttgtgccgagtccaggaacacgaccgcagataaatggccagtccggacggattgattttcattggttgatcttggatcccaatgatacagttacttttagtttcaatggggctttcatagctccaaatcgtgccagcttcttgaggggaaagtccatggggatccagagcgatgtgcaggttgatgccaattgcgaaggggaatgctaccacagtggagggactataacaagcagattgccttttcaaaacatcaatagcagagcagttggcaaatgcccaagatatgtaaaacaggaaagtttattattggcaactgggatgaagaacgttcccgaaccttccaaaaaaaggaaaaaaagaggcctgtttggcgctatagcagggtttattgaaaatggttgggaaggtctggtcgacgggtggtacggtttcaggcatcagaatgcacaaggagaaggaactgcagcagactacaaaagcacccaatcggcaattgatcagataaccggaaagttaaatagactcattgagaaaaccaaccagcaatttgagctaatagataatgaattcactgaggtggaaaagcagattggcaatttaattaactggaccaaagactccatcacagaagtatggtcttacaatgctgaacttattgtggcaatggaaaaccagcacactattgatttggctgattcagagatgaacaggctgtatgagcgagtgaggaaacaattaagggaaaatgctgaagaggatggtactggttgctttgaaatttttcataaatgtgacgatgattgtatggctagtataaggaacaatatttatgatcacagcaaatacagagaagaagcgatgcaaaatagaatacaaattgacccagtcaaattgagtagtggctacaaagatgtgatactttggtttagcttcggggcatcatgctttttgcttcttgccattgcaatgggccttgttttcatatgtgtgaagaacggaaacatgcggtgcactatttgtatataa

SEQ ID NO: 194 - protein, 454 aa, Influenza virus
MNPNQKIITIGSICLVVGLISLILQIGNIISIWISHSIQTGSQNHTGICNQNIITYKNSTWVKDTTSVILTGNSSLCPIRGWAIYSKDNSIRIGSKGDVFVIREPFISCSHLECRTFFLTQGALLNDRHSNGTVKDRSPYRALMSCPVGEAPSPYNSRFESVAWSASACHDGMGWLTIGISGPDNGAVAVLKYNGIITETIKSWRKKILRTQESECACVNGSCFTIMTDGPSDGLASYKIFKIEKGKVTKSIELNAPNSHYEECSCYPDTGKVMCVCRDNWHGSNRPWVSFDQNLDYQIGYICSGVFGDNPRPKDGTGSCGPVYVDGANGVKGFSYRYGNGVWIGRTKSHSSRHGFEMIWDPNGWTETDSKFSVRQDVVAMTDWSGYSGSFVQHPELTGLDCIRPCFWVELIRGRPKEKTIWTSASSISFCGVNSDTVDWSWPDGAELPFTIDK

SEQ ID NO: 195 - DNA, 1365 bp, Influenza virus
  source 1..1365: mol_type = other DNA
atgaatccaaatcagaaaataataaccattggatcaatctgtctggtagtcggactaattagcctaatattgcaaatagggaatataatctcaatatggattagccattcaattcaaactggaagtcaaaaccatactggaatatgcaaccaaaacatcattacctataaaaatagcacctgggtaaaggacacaacttcagtgatattaaccggcaattcatctctttgtcccatccgtgggtgggctatatacagcaaagacaatagcataagaattggttccaaaggagacgtttttgtcataagagagccctttatttcatgttctcacttggaatgcaggaccttttttctgacccaaggtgccttactgaatgacaggcattcaaatgggactgttaaggacagaagcccttatagggccttaatgagctgccctgtcggtgaagctccgtccccgtacaattcaagatttgaatcggttgcttggtcagcaagtgcatgtcatgatggcatgggctggctaacaatcggaatttcaggtccagataatggagcagtggctgtattaaaatacaacggcataataactgaaaccataaaaagttggaggaagaaaatattgaggacacaagagtctgaatgtgcctgtgtaaatggttcatgttttactataatgactgatggcccgagtgatgggctggcctcgtacaaaattttcaagatcgaaaaggggaaggttactaaatcaatagagttgaatgcacctaattctcactatgaggaatgttcctgttaccctgataccggcaaagtgatgtgtgtgtgcagagacaattggcatggttcgaaccggccatgggtgtctttcgatcaaaacctggattatcaaataggatacatctgcagtggggttttcggtgacaacccgcgtcccaaagatggaacaggcagctgtggtccagtgtatgttgatggagcaaacggagtaaagggattttcatataggtatggtaatggtgtttggataggaaggaccaaaagtcacagttccagacatgggtttgagatgatttgggatcctaatggatggacagagactgatagtaagttctctgtgaggcaagatgttgtggcaatgactgattggtcagggtatagcgggagtttcgttcaacatcctgagctaacagggctagactgtataaggccgtgcttctgggttgaattaatcaggggacgacctaaagaaaaaacaatctggactagtgcgagcagcatttctttttgtggcgtgaatagtgatactgtagattggtcttggccagacggtgctgagttgccattcaccattgacaagtag

SEQ ID NO: 196 - protein, 97 aa, Influenza virus
MSLLTEVETPTRNGWECRCNDSSDPLIIAASIIGILHLILWILNRLFFKCIYRRLKYGLKRGPSTEGVPESMREEYRQEQQSAVDVDDGHFVNIELE

SEQ ID NO: 197 - DNA, 294 bp, Influenza virus
  source 1..294: mol_type = other DNA
atgagtcttctaaccgaggttgaaacgcctaccagaaacggatgggagtgcagatgcaacgattcaagtgaccctctcattattgccgcaagtatcattgggatcttgcacttgatattgtggattcttaatcgtcttttcttcaaatgtatttatcgtcgccttaaatacggtttgaaaagagggccttctacggaaggagtgcctgagtctatgagggaagaatatcggcaggaacagcagagtgctgtggatgttgacgatggtcattttgtcaacatagagctggagtaa

SEQ ID NO: 198 - protein, 64 aa, Respiratory syncytial virus
MENTSITIEFSSKFWPYFTLIHMITTIISLLIIISIMTAILNKLCEYNVFHNKTFELPRARVNT

SEQ ID NO: 199 - DNA, 195 bp, Respiratory syncytial virus
  source 1..195: mol_type = other DNA
atggaaaacaccagcatcaccatcgagttcagcagcaagttctggccctacttcaccctgatccacatgatcaccaccatcatcagcctgctgatcatcatctccatcatgaccgccatcctgaacaagctgtgcgagtacaacgtgttccacaacaagaccttcgagctgcccagagccagagtgaacacctga

SEQ ID NO: 200 - protein, 574 aa, Respiratory syncytial virus
MELPILKANAITTILAAVTFCFASSQNITEEFYQSTCSAVSKGYLSALRTGWYTSVITIELSNIKENKCNGTDAKVKLINQELDKYKNAVTELQLLMQSTTAANNRARRELPRFMNYTLNNTKKTNVTLSKKRKRRFLGFLLGVGSAIASGIAVSKVLHLEGEVNKIKSALLSTNKAVVSLSNGVSVLTSKVLDLKNYIDKQLLPIVNKQSCRISNIETVIEFQQKNNRLLEITREFSVNAGVTTPVSTYMLTNSELLSLINDMPITNDQKKLMSNNVQIVRQQSYSIMSIIKEEVLAYVVQLPLYGVIDTPCWKLHTSPLCTTNTKEGSNICLTRTDRGWYCDNAGSVSFFPQAETCKVQSNRVFCDTMNSLTLPSEVNLCNVDIFNPKYDCKIMTSKTDVSSSVITSLGAIVSCYGKTKCTASNKNRGIIKTFSNGCDYVSNKGVDTVSVGNTLYYVNKQEGKSLYVKGEPIINFYDPLVFPSDEFDASISQVNEKINQSLAFIRKSDELLHHVNAGKSTTNIMITTIIIVIIVILLSLIAVGLLLYCKARSTPVTLSKDQLSGINNIAFSN

SEQ ID NO: 201 - DNA, 1725 bp, Respiratory syncytial virus
  source 1..1725: mol_type = other DNA
atggaactgcccatcctgaaggccaatgccatcaccacaattctggccgccgtgaccttctgctttgccagcagccagaacatcaccgaagagttctaccagagcacctgtagcgccgtgtccaagggctatctgagcgcccttagaaccggctggtacaccagcgtgatcaccatcgagctgagcaacatcaaagaaaacaagtgcaacggcaccgacgccaaagtgaagctgatcaatcaagagctggacaagtacaagaatgccgtgaccgaactgcagctgctgatgcagtctaccaccgccgccaacaacagagccagacgggaactgcctagattcatgaactacaccctgaacaacaccaaaaagaccaacgtgaccctgagcaagaagcggaagcggagattcctgggctttctgctcggagtgggaagcgccattgcctctggaatcgccgtgtctaaagtgctgcacctggaaggcgaagtgaacaagatcaagagcgccctgctgagcaccaacaaggccgtggtgtctctgagcaatggcgtgtccgtgctgaccagcaaggtgctggacctgaagaactacatcgacaaacagctgctgcccatcgtcaacaagcagagctgccggatcagcaacatcgagacagtgatcgagttccagcagaagaacaaccggctgctggaaatcacccgcgagttctctgtgaatgccggcgtgaccacacctgtgtccacctacatgctgaccaacagcgagctgctgtccctgatcaacgacatgcccatcaccaacgaccagaaaaagctgatgagcaacaacgtgcagatcgtgcggcagcagagctacagcatcatgagcattatcaaagaagaggtgctggcctacgtggtgcagctgcctctgtatggcgtgatcgataccccttgctggaagctgcacacaagccctctgtgcaccaccaataccaaagagggctccaacatctgcctgaccagaaccgacagaggctggtactgcgataatgccggcagcgtctcattcttcccacaagccgagacatgcaaggtgcagagcaaccgggtgttctgcgatacaatgaacagcctgacactgccctccgaagtgaatctgtgcaacgtggacatcttcaaccctaagtacgactgcaagatcatgacctccaagaccgacgtgtccagcagtgtgatcacctctctgggcgccatcgtgtcctgttacggcaagaccaagtgcaccgccagcaacaagaaccggggcatcatcaagaccttcagcaacggctgcgactacgtgtccaacaaaggcgtggacaccgtgtctgtgggcaacaccctgtactacgtgaacaagcaagagggcaagagcctgtacgtgaagggcgagcccatcatcaacttctacgaccctctggtgttccccagcgacgagttcgatgccagcatcagccaagtgaacgagaagatcaaccagagcctggccttcatcagaaagtccgatgagctgctgcatcacgtgaacgccggcaagtccaccaccaacatcatgatcaccaccatcattatcgtgatcatcgtcatcctgctcagcctgatcgccgtgggcctgctgctgtattgcaaggccagatctacccctgtgacactgtccaaggatcagctgagcggcatcaacaatatcgccttctccaactga

SEQ ID NO: 202 - protein, 298 aa, Respiratory syncytial virus
MSKNKDQRTAKTLEKTWDTLNHLLFISSGLYKLNLKSIAQITLSILAMIISTSLIITAIIFIASANHKVTLTTAIIQDATSQIKNTTPTYLTQDPQLGISFSNLSEITSQTTTILASTTPGVKSNLQPTTVKTKNTTTTQTQPSKPTTKQRQNKPPNKPNNDFHFEVFNFVPCSICSNNPTCWAICKRIPNKKPGKKTTTKPTKKPTFKTTKKDLKPQTTKPKEVPTTKPTEEPTINTTKTNITTTLLTNNTTGNPKLTSQMETFHSTSSEGNLSPSQVSTTSEHPSQPSSPPNTTRQ

SEQ ID NO: 203 - DNA, 897 bp, Respiratory syncytial virus
  source 1..897: mol_type = other DNA
atgagcaagaacaaggaccagcggaccgccaagacactggaaaagacctgggacaccctgaaccatctgctgttcatcagcagcggcctgtacaagctgaacctgaagtctatcgcccagatcaccctgagcatcctggccatgatcatcagcaccagcctgatcatcaccgccatcatctttatcgccagcgccaaccacaaagtgaccctgaccacagccatcatccaggacgccacaagccagatcaagaacaccacacctacctacctgacacaggaccctcagctgggcatcagcttcagcaacctgagcgagatcaccagccagaccaccaccattctggccagcacaacccctggcgtgaagtccaatctgcagcccaccaccgtgaaaacaaagaacacaaccaccacacagacccagcctagcaagcctaccaccaagcagcggcagaacaagcctcctaacaagcccaacaacgacttccacttcgaggtgttcaacttcgtgccctgcagcatctgcagcaacaaccctacctgttgggccatctgcaagcggatccccaacaagaagcccggcaagaaaaccaccactaagcccacaaagaagcccaccttcaagaccaccaagaaggacctgaagcctcagaccacaaagcccaaagaggtgcccaccacaaaacccaccgaggaacccaccatcaacacaacaaagaccaacatcaccaccacgctgctgaccaacaataccaccggcaatcccaagctgacctctcagatggaaaccttccacagcacctccagcgagggcaatctgagcccttctcaggtgtccacaaccagcgagcaccctagccagccaagctctcctcctaacaccacacggcagtag

SEQ ID NO: 204 - DNA, 14 bp, synthetic construct
  source 1..14: mol_type = other DNA
aatagatcgttgtc

SEQ ID NO: 205 - DNA, 16 bp, synthetic construct
  source 1..16: mol_type = other DNA
gatctatagatctgtc

SEQ ID NO: 206 - DNA, 14 bp, synthetic construct
  source 1..14: mol_type = other DNA
ttgtatctgtatta